European Patent Specification EP 3 169 309 B1, published May 10, 2023. Title: METHOD OF ENCAPSULATING A NUCLEIC ACID IN A LIPID NANOPARTICLE HOST. Applicant: NOVARTIS AG. Application PCT/US2015/039879. The sequence listing filed with the application follows.

SEQUENCE LISTING (11 sequences)

SEQ ID NO: 1 - DNA, 18 bp, Artificial Sequence
  siRNA antisense strand; APOC3 gene
agcactgagaatactgtc

SEQ ID NO: 2 - DNA, 18 bp, Artificial Sequence
  siRNA antisense strand; APOC3 gene
ttcttgtccagctttatt

SEQ ID NO: 3 - DNA, 18 bp, Artificial Sequence
  siRNA antisense strand; APOC3 gene
acaacaaggagtacccgg

SEQ ID NO: 4 - DNA, 21 bp, Artificial Sequence
  siRNA antisense strand; FVII gene
uuuaauugaaaccaagacauu

SEQ ID NO: 5 - DNA, 21 bp, Artificial Sequence
  siRNA antisense strand; EPAS1 gene
ucaugaaaucguuacguuguu

SEQ ID NO: 6 - RNA, 1080 nt, Artificial Sequence
  TEV-hLeptin-GAopt-2xhBG-120A
  5'UTR (14)..(154): Tobacco Etch Virus (TEV) 5' UTR: 14-154
  misc_feature (155)..(163): Optimal Kozak sequence
  3'UTR (689)..(954): 2 copies of human beta-globin 3'UTR: 689-954
  polyA_signal (961)..(1080)
gggagacgcguguuaaauaacaaaucucaacacaacauauacaaaacaaacgaaucucaagcaaucaagcauucuacuucuauugcagcaauuuaaaucauuucuuuuaaagcaaaagcaauuuucugaaaauuuucaccauuuacgaacgauagccgccaccaugcacuggggaacccugugcggauuccuguggcuguggcccuaccuguucuaugugcaagccgugcccauccagaaggugcaggacgacaccaagacccugaucaagaccaucgugacccggaucaacgacaucagccacacccagagcguguccagcaagcagaaagugaccggccuggacuucauccccggccugcacccuauccugacccuguccaagauggaccagacccuggccguguaccagcagauccugaccagcaugcccagccggaacgugauccagaucagcaacgaccuggaaaaccugcgggaccugcugcacgugcuggccuucagcaagagcugccaucugccuugggccagcggccuggaaacccuggauucucugggcggagugcuggaagccagcggcuacucuacagaggugguggcccugagcagacugcagggcagccugcaggauaugcuguggcagcuggaucugagccccggcugcuaauagcggaccggcgauagaugaagcucgcuuucuugcuguccaauuucuauuaaagguuccuuuguucccuaaguccaacuacuaaacugggggauauuaugaagggccuugagcaucuggauucugccuaauaaaaaacauuuauuuucauugcagcucgcuuucuugcuguccaauuucuauuaaagguuccuuuguucccuaaguccaacuacuaaacugggggauauuaugaagggccuugagcaucuggauucugccuaauaaaaaacauuuauuuucauugcggccgcaaaaaaaaaaaaaaaaaaaaaaaaaaaaaaaaaaaaaaaaaaaaaaaaaaaaaaaaaaaaaaaaaaaaaaaaaaaaaaaaaaaaaaaaaaaaaaaaaaaaaaaaaaaaaaaaaaaaaaaa

SEQ ID NO: 7 - DNA, 18 bp, Artificial Sequence
  siRNA sense strand; APOC3 gene
gacagtattctcagtgct

SEQ ID NO: 8 - DNA, 18 bp, Artificial Sequence
  siRNA sense strand; APOC3 gene
aataaagctggacaagaa

SEQ ID NO: 9 - DNA, 18 bp, Artificial Sequence
  siRNA sense strand; APOC3 gene
ccgggtactccttgttgt

SEQ ID NO: 10 - DNA, 21 bp, Artificial Sequence
  siRNA sense strand; FVII gene
ugucuugguuucaauuaaauu

SEQ ID NO: 11 - DNA, 21 bp, Artificial Sequence
  siRNA sense strand; EPAS1 gene
caacguaacgauuucaugauu